European Patent Specification EP 3 773 551 B1, published October 16, 2024. Title: COMPOUNDS WITH ANTI-TUMOR ACTIVITY AGAINST CANCER CELLS BEARING HER2 EXON 19 MUTATIONS. Applicant: Board of Regents, The University of Texas System. The sequence listing filed with the application follows.

SEQUENCE LISTING (1 sequence)

SEQ ID NO: 1 - protein, 102 aa, Homo sapiens
GVVFGILIKRRQQKIRKYTMRRLLQETELVEPLTPSGAMPNQAQMRILKETELRKVKVLGSGAFGTVYKGIWIPDGENVKIPVAIKVLRENTSPKANKEILD